European Patent Application EP 4 321 526 A1, published February 14, 2024. Title: 탄산탈수소효소 IX를 표적으로 하는 펩타이드 리간드, 이를 포함하는 펩타이드 구조체 및 이 들의 용도. Applicant: (주)씨바이오멕스. Application KR. The sequence listing filed with the application follows.

SEQUENCE LISTING (44 sequences)

SEQ ID NO: 1 - protein, 7 aa, synthetic construct
  REGION 1..7: note = Synthetic Polypeptide
  REGION 1..7: note = MISC_FEATURE - L-amino acid residue or D-amino acid residue
RAHKHYH

SEQ ID NO: 2 - protein, 7 aa, synthetic construct
  REGION 1..7: note = Synthetic Polypeptide
  REGION 1..7: note = MISC_FEATURE - L-amino acid residue or D-amino acid residue
HRKHDDN

SEQ ID NO: 3 - protein, 7 aa, synthetic construct
  REGION 1..7: note = Synthetic Polypeptide
  REGION 1..7: note = MISC_FEATURE - L-amino acid residue or D-amino acid residue
AYYRKKW

SEQ ID NO: 4 - protein, 7 aa, synthetic construct
  REGION 1..7: note = Synthetic Polypeptide
  REGION 1..7: note = MISC_FEATURE - L-amino acid residue or D-amino acid residue
RRLLFSG

SEQ ID NO: 5 - protein, 7 aa, synthetic construct
  REGION 1..7: note = Synthetic Polypeptide
  REGION 1..7: note = MISC_FEATURE - L-amino acid residue or D-amino acid residue
RRFHFTH

SEQ ID NO: 6 - protein, 7 aa, synthetic construct
  REGION 1..7: note = Synthetic Polypeptide
  REGION 1..7: note = MISC_FEATURE - L-amino acid residue or D-amino acid residue
FHSRRDV

SEQ ID NO: 7 - protein, 7 aa, synthetic construct
  REGION 1..7: note = Synthetic Polypeptide
  REGION 1..7: note = MISC_FEATURE - L-amino acid residue or D-amino acid residue
VLRNKSD

SEQ ID NO: 8 - protein, 7 aa, synthetic construct
  REGION 1..7: note = Synthetic Polypeptide
  REGION 1..7: note = MISC_FEATURE - L-amino acid residue or D-amino acid residue
RSRHFHY

SEQ ID NO: 9 - protein, 7 aa, synthetic construct
  REGION 1..7: note = Synthetic Polypeptide
  REGION 1..7: note = MISC_FEATURE - L-amino acid residue or D-amino acid residue
FHRIKHL

SEQ ID NO: 10 - protein, 7 aa, synthetic construct
  REGION 1..7: note = Synthetic Polypeptide
  REGION 1..7: note = MISC_FEATURE - L-amino acid residue or D-amino acid residue
RITAINY

SEQ ID NO: 11 - protein, 7 aa, synthetic construct
  REGION 1..7: note = Synthetic Polypeptide
  REGION 1..7: note = MISC_FEATURE - L-amino acid residue or D-amino acid residue
YHKHIRQ

SEQ ID NO: 12 - protein, 7 aa, synthetic construct
  REGION 1..7: note = Synthetic Polypeptide
  REGION 1..7: note = MISC_FEATURE - L-amino acid residue or D-amino acid residue
HFVKKFR

SEQ ID NO: 13 - protein, 7 aa, synthetic construct
  REGION 1..7: note = Synthetic Polypeptide
  REGION 1..7: note = MISC_FEATURE - L-amino acid residue or D-amino acid residue
FFKRKHE

SEQ ID NO: 14 - protein, 7 aa, synthetic construct
  REGION 1..7: note = Synthetic Polypeptide
  REGION 1..7: note = MISC_FEATURE - L-amino acid residue or D-amino acid residue
HGHLFKR

SEQ ID NO: 15 - protein, 7 aa, synthetic construct
  REGION 1..7: note = Synthetic Polypeptide
  REGION 1..7: note = MISC_FEATURE - L-amino acid residue or D-amino acid residue
RFHHFRN

SEQ ID NO: 16 - protein, 7 aa, synthetic construct
  REGION 1..7: note = Synthetic Polypeptide
  REGION 1..7: note = MISC_FEATURE - L-amino acid residue or D-amino acid residue
RLSKFHS

SEQ ID NO: 17 - protein, 7 aa, synthetic construct
  REGION 1..7: note = Synthetic Polypeptide
  REGION 1..7: note = MISC_FEATURE - L-amino acid residue or D-amino acid residue
YETFRTR

SEQ ID NO: 18 - protein, 7 aa, synthetic construct
  REGION 1..7: note = Synthetic Polypeptide
  REGION 1..7: note = MISC_FEATURE - L-amino acid residue or D-amino acid residue
RRFRHYH

SEQ ID NO: 19 - protein, 7 aa, synthetic construct
  REGION 1..7: note = Synthetic Polypeptide
  REGION 1..7: note = MISC_FEATURE - L-amino acid residue or D-amino acid residue
  SITE 3: note = MISC_FEATURE - Xaa is 3-(1-naphthyl)-alanine
RRXRHKH

SEQ ID NO: 20 - protein, 7 aa, synthetic construct
  REGION 1..7: note = Synthetic Polypeptide
  REGION 1..7: note = MISC_FEATURE - L-amino acid residue or D-amino acid residue
HYHRFRR

SEQ ID NO: 21 - protein, 7 aa, synthetic construct
  REGION 1..7: note = Synthetic Polypeptide
  REGION 1..7: note = MISC_FEATURE - L-amino acid residue or D-amino acid residue
  SITE 2: note = MISC_FEATURE - Xaa is 2,3,4,5,6-pentafluoro-phenylalanine
HXHRFRR

SEQ ID NO: 22 - protein, 7 aa, synthetic construct
  REGION 1..7: note = Synthetic Polypeptide
  REGION 1..7: note = MISC_FEATURE - L-amino acid residue or D-amino acid residue
  SITE 2: note = MISC_FEATURE - Xaa is 4-amino-phenylalanine
HXHRFRR

SEQ ID NO: 23 - protein, 7 aa, synthetic construct
  REGION 1..7: note = Synthetic Polypeptide
  REGION 1..7: note = MISC_FEATURE - L-amino acid residue or D-amino acid residue
  SITE 2: note = MISC_FEATURE - Xaa is 3-(1-naphthyl)-alanine
HXHRFRR

SEQ ID NO: 24 - protein, 7 aa, synthetic construct
  REGION 1..7: note = Synthetic Polypeptide
  REGION 1..7: note = MISC_FEATURE - L-amino acid residue or D-amino acid residue
  SITE 2: note = MISC_FEATURE - Xaa is 4-phenyl-phenylalanine
HXHRFRR

SEQ ID NO: 25 - protein, 7 aa, synthetic construct
  REGION 1..7: note = Synthetic Polypeptide
  REGION 1..7: note = MISC_FEATURE - L-amino acid residue or D-amino acid residue
  SITE 5: note = MISC_FEATURE - Xaa is 2,3,4,5,6-pentafluoro-phenylalanine
HYHRXRR

SEQ ID NO: 26 - protein, 7 aa, synthetic construct
  REGION 1..7: note = Synthetic Polypeptide
  REGION 1..7: note = MISC_FEATURE - L-amino acid residue or D-amino acid residue
  SITE 5: note = MISC_FEATURE - Xaa is 4-amino-phenylalanine
HYHRXRR

SEQ ID NO: 27 - protein, 7 aa, synthetic construct
  REGION 1..7: note = Synthetic Polypeptide
  REGION 1..7: note = MISC_FEATURE - L-amino acid residue or D-amino acid residue
  SITE 5: note = MISC_FEATURE - Xaa is 3-(1-naphthyl)-alanine
HYHRXRR

SEQ ID NO: 28 - protein, 7 aa, synthetic construct
  REGION 1..7: note = Synthetic Polypeptide
  REGION 1..7: note = MISC_FEATURE - L-amino acid residue or D-amino acid residue
  SITE 5: note = MISC_FEATURE - Xaa is 4-phenyl-phenylalanine
HYHRXRR

SEQ ID NO: 29 - protein, 5 aa, synthetic construct
  REGION 1..5: note = Synthetic Polypeptide
  REGION 1..5: note = MISC_FEATURE - L-amino acid residue or D-amino acid residue
RRFRY

SEQ ID NO: 30 - protein, 5 aa, synthetic construct
  REGION 1..5: note = Synthetic Polypeptide
  REGION 1..5: note = MISC_FEATURE - L-amino acid residue or D-amino acid residue
  SITE 3: note = MISC_FEATURE - Xaa is 3-(1-naphthyl)-alanine
RRXRY

SEQ ID NO: 31 - protein, 5 aa, synthetic construct
  REGION 1..5: note = Synthetic Polypeptide
  REGION 1..5: note = MISC_FEATURE - L-amino acid residue or D-amino acid residue
RRFRK

SEQ ID NO: 32 - protein, 5 aa, synthetic construct
  REGION 1..5: note = Synthetic Polypeptide
  REGION 1..5: note = MISC_FEATURE - L-amino acid residue or D-amino acid residue
  SITE 3: note = MISC_FEATURE - Xaa is 3-(1-naphthyl)-alanine
RRXRK

SEQ ID NO: 33 - protein, 5 aa, synthetic construct
  REGION 1..5: note = Synthetic Polypeptide
  REGION 1..5: note = MISC_FEATURE - L-amino acid residue or D-amino acid residue
  SITE 3: note = MISC_FEATURE - Xaa is 3-(1-naphthyl)-alanine
ERXRK

SEQ ID NO: 34 - protein, 5 aa, synthetic construct
  REGION 1..5: note = Synthetic Polypeptide
  REGION 1..5: note = MISC_FEATURE - L-amino acid residue or D-amino acid residue
  SITE 3: note = MISC_FEATURE - Xaa is 3-(1-naphthyl)-alanine
RRXEK

SEQ ID NO: 35 - protein, 5 aa, synthetic construct
  REGION 1..5: note = Synthetic Polypeptide
  REGION 1..5: note = MISC_FEATURE - L-amino acid residue or D-amino acid residue
  SITE 3: note = MISC_FEATURE - Xaa is homo-phenylalanine
RRXRY

SEQ ID NO: 36 - protein, 5 aa, synthetic construct
  REGION 1..5: note = Synthetic Polypeptide
  REGION 1..5: note = MISC_FEATURE - L-amino acid residue or D-amino acid residue
  SITE 3: note = MISC_FEATURE - Xaa is 3-(1-naphthyl)-alanine
ERXEK

SEQ ID NO: 37 - protein, 5 aa, synthetic construct
  REGION 1..5: note = Synthetic Polypeptide
  REGION 1..5: note = MISC_FEATURE - L-amino acid residue or D-amino acid residue
YRFRR

SEQ ID NO: 38 - protein, 5 aa, synthetic construct
  REGION 1..5: note = Synthetic Polypeptide
  REGION 1..5: note = MISC_FEATURE - L-amino acid residue or D-amino acid residue
YEFRR

SEQ ID NO: 39 - protein, 5 aa, synthetic construct
  REGION 1..5: note = Synthetic Polypeptide
  REGION 1..5: note = MISC_FEATURE - L-amino acid residue or D-amino acid residue
YRFER

SEQ ID NO: 40 - protein, 5 aa, synthetic construct
  REGION 1..5: note = Synthetic Polypeptide
  REGION 1..5: note = MISC_FEATURE - L-amino acid residue or D-amino acid residue
YRFRE

SEQ ID NO: 41 - protein, 5 aa, synthetic construct
  REGION 1..5: note = Synthetic Polypeptide
  REGION 1..5: note = MISC_FEATURE - L-amino acid residue or D-amino acid residue
  SITE 3: note = MISC_FEATURE - Xaa is 3-(1-naphthyl)-alanine
KRXRR

SEQ ID NO: 42 - protein, 5 aa, synthetic construct
  REGION 1..5: note = Synthetic Polypeptide
  REGION 1..5: note = MISC_FEATURE - L-amino acid residue or D-amino acid residue
  SITE 3: note = MISC_FEATURE - Xaa is 3-(1-naphthyl)-alanine
YRXRR

SEQ ID NO: 43 - protein, 5 aa, synthetic construct
  REGION 1..5: note = Synthetic Polypeptide
  REGION 1..5: note = MISC_FEATURE - L-amino acid residue or D-amino acid residue
KRFRR

SEQ ID NO: 44 - skipped